European Patent Application EP 4 116 440 A1, published January 11, 2023. Title: RT-PCR Detection Method and Kit For Novel Coronavirus. Applicant: Daan Gene Co., Ltd. The sequence listing filed with the application follows.

SEQUENCE LISTING (10 sequences)

SEQ ID NO: 1 - DNA, 19 bp, Artificial sequence
  Primer
ttttcttgctttcgtggta

SEQ ID NO: 2 - DNA, 20 bp, Artificial sequence
  Primer
ggttttacaagactcacgtt

SEQ ID NO: 3 - DNA, 20 bp, Artificial sequence
  Probe
attgcagcagtacgcacaca

SEQ ID NO: 4 - DNA, 22 bp, Artificial sequence
  Primer
caagtaagtttctccgaatccc

SEQ ID NO: 5 - DNA, 19 bp, Artificial sequence
  Primer
gctgaagtcccatgaccgt

SEQ ID NO: 6 - DNA, 25 bp, Artificial sequence
  Probe
caactggaggtagagacggactgcg

SEQ ID NO: 7 - DNA, 20 bp, Artificial sequence
  Primer
ctttcgtggtattcttgcta

SEQ ID NO: 8 - DNA, 21 bp, Artificial sequence
  Primer
ctcacgttaacaatattgcag

SEQ ID NO: 9 - DNA, 19 bp, Artificial sequence
  Primer
agttacactagccatcctt

SEQ ID NO: 10 - DNA, 21 bp, Artificial sequence
  Primer
tttaacacgagagtaaacgta